European Patent Specification EP 3 468 584 B1, published May 31, 2023. Title: COMBINATORIAL ANDROGEN DEPRIVATION WITH AN ANDROGEN RECEPTOR VACCINE. Applicant: WISCONSIN ALUMNI RESEARCH FOUNDATION McNeel, Douglas Olsen, Brian. The sequence listing filed with the application follows.

SEQUENCE LISTING (20 sequences)

SEQ ID NO: 1 - DNA, 10070 bp, Homo sapiens
gcggagagaaccctctgttttcccccactctctctccacctcctcctgccttccccaccccgagtgcggagccagagatcaaaagatgaaaaggcagtcaggtcttcagtagccaaaaaacaaaacaaacaaaaacaaaaaagccgaaataaaagaaaaagataataactcagttcttatttgcacctacttcagtggacactgaatttggaaggtggaggattttgtttttttcttttaagatctgggcatcttttgaatctacccttcaagtattaagagacagactgtgagcctagcagggcagatcttgtccaccgtgtgtcttcttctgcacgagactttgaggctgtcagagcgctttttgcgtggttgctcccgcaagtttccttctctggagcttcccgcaggtgggcagctagctgcagcgactaccgcatcatcacagcctgttgaactcttctgagcaagagaaggggaggcggggtaagggaagtaggtggaagattcagccaagctcaaggatggaagtgcagttagggctgggaagggtctaccctcggccgccgtccaagacctaccgaggagctttccagaatctgttccagagcgtgcgcgaagtgatccagaacccgggccccaggcacccagaggccgcgagcgcagcacctcccggcgccagtttgctgctgctgcagcagcagcagcagcagcagcagcagcagcagcagcagcagcagcagcagcagcagcagcagcagcaagagactagccccaggcagcagcagcagcagcagggtgaggatggttctccccaagcccatcgtagaggccccacaggctacctggtcctggatgaggaacagcaaccttcacagccgcagtcggccctggagtgccaccccgagagaggttgcgtcccagagcctggagccgccgtggccgccagcaaggggctgccgcagcagctgccagcacctccggacgaggatgactcagctgccccatccacgttgtccctgctgggccccactttccccggcttaagcagctgctccgctgaccttaaagacatcctgagcgaggccagcaccatgcaactccttcagcaacagcagcaggaagcagtatccgaaggcagcagcagcgggagagcgagggaggcctcgggggctcccacttcctccaaggacaattacttagggggcacttcgaccatttctgacaacgccaaggagttgtgtaaggcagtgtcggtgtccatgggcctgggtgtggaggcgttggagcatctgagtccaggggaacagcttcggggggattgcatgtacgccccacttttgggagttccacccgctgtgcgtcccactccttgtgccccattggccgaatgcaaaggttctctgctagacgacagcgcaggcaagagcactgaagatactgctgagtattcccctttcaagggaggttacaccaaagggctagaaggcgagagcctaggctgctctggcagcgctgcagcagggagctccgggacacttgaactgccgtctaccctgtctctctacaagtccggagcactggacgaggcagctgcgtaccagagtcgcgactactacaactttccactggctctggccggaccgccgccccctccgccgcctccccatccccacgctcgcatcaagctggagaacccgctggactacggcagcgcctgggcggctgcggcggcgcagtgccgctatggggacctggcgagcctgcatggcgcgggtgcagcgggacccggttctgggtcaccctcagccgccgcttcctcatcctggcacactctcttcacagccgaagaaggccagttgtatggaccgtgtggtggtggtgggggtggtggcggcggcggcggcggcggcggcggcggcggcggcggcggcggcggcggcgaggcgggagctgtagccccctacggctacactcggccccctcaggggctggcgggccaggaaagcgacttcaccgcacctgatgtgtggtaccctggcggcatggtgagcagagtgccctatcccagtcccacttgtgtcaaaagcgaaatgggcccctggatggatagctactccggaccttacggggacatgcgtttggagactgccagggaccatgttttgcccattgactattactttccaccccagaagacctgcctgatctgtggagatgaagcttctgggtgtcactatggagctctcacatgtggaagctgcaaggtcttcttcaaaagagccgctgaagggaaacagaagtacctgtgcgccagcagaaatgattgcactattgataaattccgaaggaaaaattgtccatcttgtcgtcttcggaaatgttatgaagcagggatgactctgggagcccggaagctgaagaaacttggtaatctgaaactacaggaggaaggagaggcttccagcaccaccagccccactgaggagacaacccagaagctgacagtgtcacacattgaaggctatgaatgtcagcccatctttctgaatgtcctggaagccattgagccaggtgtagtgtgtgctggacacgacaacaaccagcccgactcctttgcagccttgctctctagcctcaatgaactgggagagagacagcttgtacacgtggtcaagtgggccaaggccttgcctggcttccgcaacttacacgtggacgaccagatggctgtcattcagtactcctggatggggctcatggtgtttgccatgggctggcgatccttcaccaatgtcaactccaggatgctctacttcgcccctgatctggttttcaatgagtaccgcatgcacaagtcccggatgtacagccagtgtgtccgaatgaggcacctctctcaagagtttggatggctccaaatcaccccccaggaattcctgtgcatgaaagcactgctactcttcagcattattccagtggatgggctgaaaaatcaaaaattctttgatgaacttcgaatgaactacatcaaggaactcgatcgtatcattgcatgcaaaagaaaaaatcccacatcctgctcaagacgcttctaccagctcaccaagctcctggactccgtgcagcctattgcgagagagctgcatcagttcacttttgacctgctaatcaagtcacacatggtgagcgtggactttccggaaatgatggcagagatcatctctgtgcaagtgcccaagatcctttctgggaaagtcaagcccatctatttccacacccagtgaagcattggaaaccctatttccccaccccagctcatgccccctttcagatgtcttctgcctgttataactctgcactactcctctgcagtgccttggggaatttcctctattgatgtacagtctgtcatgaacatgttcctgaattctatttgctgggctttttttttctctttctctcctttctttttcttcttccctccctatctaaccctcccatggcaccttcagactttgcttcccattgtggctcctatctgtgttttgaatggtgttgtatgcctttaaatctgtgatgatcctcatatggcccagtgtcaagttgtgcttgtttacagcactactctgtgccagccacacaaacgtttacttatcttatgccacgggaagtttagagagctaagattatctggggaaatcaaaacaaaaacaagcaaacaaaaaaaaaaagcaaaaacaaaacaaaaaataagccaaaaaaccttgctagtgttttttcctcaaaaataaataaataaataaataaatacgtacatacatacacacatacatacaaacatatagaaatccccaaagaggccaatagtgacgagaaggtgaaaattgcaggcccatggggagttactgattttttcatctcctccctccacgggagactttattttctgccaatggctattgccattagagggcagagtgaccccagagctgagttgggcaggggggtggacagagaggagaggacaaggagggcaatggagcatcagtacctgcccacagccttggtccctgggggctagactgctcaactgtggagcaattcattatactgaaaatgtgcttgttgttgaaaatttgtctgcatgttaatgcctcacccccaaacccttttctctctcactctctgcctccaacttcagattgactttcaatagtttttctaagacctttgaactgaatgttctcttcagccaaaacttggcgacttccacagaaaagtctgaccactgagaagaaggagagcagagatttaaccctttgtaaggccccatttggatccaggtctgctttctcatgtgtgagtcagggaggagctggagccagaggagaagaaaatgatagcttggctgttctcctgcttaggacactgactgaatagttaaactctcactgccactaccttttccccacctttaaaagacctgaatgaagttttctgccaaactccgtgaagccacaagcaccttatgtcctcccttcagtgttttgtgggcctgaatttcatcacactgcatttcagccatggtcatcaagcctgtttgcttcttttgggcatgttcacagattctctgttaagagcccccaccaccaagaaggttagcaggccaacagctctgacatctatctgtagatgccagtagtcacaaagatttcttaccaactctcagatcgctggagcccttagacaaactggaaagaaggcatcaaagggatcaggcaagctgggcgtcttgcccttgtcccccagagatgataccctcccagcaagtggagaagttctcacttccttctttagagcagctaaaggggctacccagatcagggttgaagagaaaactcaattaccagggtgggaagaatgaaggcactagaaccagaaaccctgcaaatgctcttcttgtcacccagcatatccacctgcagaagtcatgagaagagagaaggaacaaagaggagactctgactactgaattaaaatcttcagcggcaaagcctaaagccagatggacaccatctggtgagtttactcatcatcctcctctgctgctgattctgggctctgacattgcccatactcactcagattccccacctttgttgctgcctcttagtcagagggaggccaaaccattgagactttctacagaaccatggcttctttcggaaaggtctggttggtgtggctccaatactttgccacccatgaactcagggtgtgccctgggacactggttttatatagtcttttggcacacctgtgttctgttgacttcgttcttcaagcccaagtgcaagggaaaatgtccacctactttctcatcttggcctctgcctccttacttagctcttaatctcatctgttgaactcaagaaatcaagggccagtcatcaagctgcccattttaattgattcactctgtttgttgagaggatagtttctgagtgacatgatatgatccacaagggtttccttccctgatttctgcattgatattaatagccaaacgaacttcaaaacagctttaaataacaagggagaggggaacctaagatgagtaatatgccaatccaagactgctggagaaaactaaagctgacaggttccctttttggggtgggatagacatgttctggttttctttattattacacaatctggctcatgtacaggatcacttttagctgttttaaacagaaaaaaatatccaccactcttttcagttacactaggttacattttaataggtcctttacatctgttttggaatgattttcatcttttgtgatacacagattgaattatatcattttcatatctctccttgtaaatactagaagctctcctttacatttctctatcaaatttttcatctttatgggtttcccaattgtgactcttgtcttcatgaatatatgtttttcatttgcaaaagccaaaaatcagtgaaacagcagtgtaattaaaagcaacaactggattactccaaatttccaaatgacaaaactagggaaaaatagcctacacaagcctttaggcctactctttctgtgcttgggtttgagtgaacaaaggagattttagcttggctctgttctcccatggatgaaaggaggaggattttttttttcttttggccattgatgttctagccaatgtaattgacagaagtctcattttgcatgcgctctgctctacaaacagagttggtatggttggtatactgtactcacctgtgagggactggccactcagacccacttagctggtgagctagaagatgaggatcactcactggaaaagtcacaaggaccatctccaaacaagttggcagtgctcgatgtggacgaagagtgaggaagagaaaaagaaggagcaccagggagaaggctccgtctgtgctgggcagcagacagctgccaggatcacgaactctgtagtcaaagaaaagagtcgtgtggcagtttcagctctcgttcattgggcagctcgcctaggcccagcctctgagctgacatgggagttgttggattctttgtttcatagctttttctatgccataggcaatattgttgttcttggaaagtttattatttttttaactcccttactctgagaaagggatattttgaaggactgtcatatatctttgaaaaaagaaaatctgtaatacatatatttttatgtatgttcactggcactaaaaaatatagagagcttcattctgtcctttgggtagttgctgaggtaattgtccaggttgaaaaataatgtgctgatgctagagtccctctctgtccatactctacttctaaatacatataggcatacatagcaagttttatttgacttgtactttaagagaaaatatgtccaccatccacatgatgcacaaatgagctaacattgagcttcaagtagcttctaagtgtttgtttcattaggcacagcacagatgtggcctttccccccttctctcccttgatatctggcagggcataaaggcccaggccacttcctctgccccttcccagccctgcaccaaagctgcatttcaggagactctctccagacagcccagtaactacccgagcatggcccctgcatagccctggaaaaataagaggctgactgtctacgaattatcttgtgccagttgcccaggtgagagggcactgggccaagggagtggttttcatgtttgacccactacaaggggtcatgggaatcaggaatgccaaagcaccagatcaaatccaaaacttaaagtcaaaataagccattcagcatgttcagtttcttggaaaaggaagtttctacccctgatgcctttgtaggcagatctgttctcaccattaatctttttgaaaatcttttaaagcagtttttaaaaagagagatgaaagcatcacattatataaccaaagattacattgtacctgctaagataccaaaattcataagggcagggggggagcaagcattagtgcctctttgataagctgtccaaagacagactaaaggactctgctggtgactgacttataagagctttgtgggtttttttttccctaataatatacatgtttagaagaattgaaaataatttcgggaaaatgggattatgggtccttcactaagtgattttataagcagaactggctttccttttctctagtagttgctgagcaaattgttgaagctccatcattgcatggttggaaatggagctgttcttagccactgtgtttgctagtgcccatgttagcttatctgaagatgtgaaacccttgctgataagggagcatttaaagtactagattttgcactagagggacagcaggcagaaatccttatttctgcccactttggatggcacaaaaagttatctgcagttgaaggcagaaagttgaaatacattgtaaatgaatatttgtatccatgtttcaaaattgaaatatatatatatatatatatatatatatatatatatatatagtgtgtgtgtgtgttctgatagctttaactttctctgcatctttatatttggttccagatcacacctgatgccatgtacttgtgagagaggatgcagttttgttttggaagctctctcagaacaaacaagacacctggattgatcagttaactaaaagttttctcccctattgggtttgacccacaggtcctgtgaaggagcagagggataaaaagagtagaggacatgatacattgtactttactagttcaagacagatgaatgtggaaagcataaaaactcaatggaactgactgagatttaccacagggaaggcccaaacttggggccaaaagcctacccaagtgattgaccagtggccccctaatgggacctgagctgttggaagaagagaactgttccttggtcttcaccatccttgtgagagaagggcagtttcctgcattggaacctggagcaagcgctctatctttcacacaaattccctcacctgagattgaggtgctcttgttactgggtgtctgtgtgctgtaattctggttttggatatgttctgtaaagattttgacaaatgaaaatgtgtttttctctgttaaaacttgtcagagtactagaagttgtatctctgtaggtgcaggtccatttctgcccacaggtagggtgtttttctttgattaagagattgacacttctgttgcctaggacctcccaactcaaccatttctaggtgaaggcagaaaaatccacattagttactcctcttcagacatttcagctgagataacaaatcttttggaattttttcacccatagaaagagtggtagatatttgaatttagcaggtggagtttcatagtaaaaacagcttttgactcagctttgatttatcctcatttgatttggccagaaagtaggtaatatgcattgattggcttctgattccaattcagtatagcaaggtgctaggttttttcctttccccacctgtctcttagcctggggaattaaatgagaagccttagaatgggtggcccttgtgacctgaaacacttcccacataagctacttaacaagattgtcatggagctgcagattccattgcccaccaaagactagaacacacacatatccatacaccaaaggaaagacaattctgaaatgctgtttctctggtggttccctctctggctgctgcctcacagtatgggaacctgtactctgcagaggtgacaggccagatttgcattatctcacaaccttagcccttggtgctaactgtcctacagtgaagtgcctggggggttgtcctatcccataagccacttggatgctgacagcagccaccatcagaatgacccacgcaaaaaaaagaaaaaaaaaattaaaaagtcccctcacaacccagtgacacctttctgctttcctctagactggaacattgattagggagtgcctcagacatgacattcttgtgctgtccttggaattaatctggcagcaggagggagcagactatgtaaacagagataaaaattaattttcaatattgaaggaaaaaagaaataagaagagagagagaaagaaagcatcacacaaagattttcttaaaagaaacaattttgcttgaaatctctttagatggggctcatttctcacggtggcacttggcctccactgggcagcaggaccagctccaagcgctagtgttctgttctctttttgtaatcttggaatcttttgttgctctaaatacaattaaaaatggcagaaacttgtttgttggactacatgtgtgactttgggtctgtctctgcctctgctttcagaaatgtcatccattgtgtaaaatattggcttactggtctgccagctaaaacttggccacatcccctgttatggctgcaggatcgagttattgttaacaaagagacccaagaaaagctgctaatgtcctcttatcattgttgttaatttgttaaaacataaagaaatctaaaatttcaaaaaa

SEQ ID NO: 2 - protein, 920 aa, Homo sapiens
MEVQLGLGRVYPRPPSKTYRGAFQNLFQSVREVIQNPGPRHPEAASAAPPGASLLLLQQQQQQQQQQQQQQQQQQQQQQQETSPRQQQQQQGEDGSPQAHRRGPTGYLVLDEEQQPSQPQSALECHPERGCVPEPGAAVAASKGLPQQLPAPPDEDDSAAPSTLSLLGPTFPGLSSCSADLKDILSEASTMQLLQQQQQEAVSEGSSSGRAREASGAPTSSKDNYLGGTSTISDNAKELCKAVSVSMGLGVEALEHLSPGEQLRGDCMYAPLLGVPPAVRPTPCAPLAECKGSLLDDSAGKSTEDTAEYSPFKGGYTKGLEGESLGCSGSAAAGSSGTLELPSTLSLYKSGALDEAAAYQSRDYYNFPLALAGPPPPPPPPHPHARIKLENPLDYGSAWAAAAAQCRYGDLASLHGAGAAGPGSGSPSAAASSSWHTLFTAEEGQLYGPCGGGGGGGGGGGGGGGGGGGGGGGEAGAVAPYGYTRPPQGLAGQESDFTAPDVWYPGGMVSRVPYPSPTCVKSEMGPWMDSYSGPYGDMRLETARDHVLPIDYYFPPQKTCLICGDEASGCHYGALTCGSCKVFFKRAAEGKQKYLCASRNDCTIDKFRRKNCPSCRLRKCYEAGMTLGARKLKKLGNLKLQEEGEASSTTSPTEETTQKLTVSHIEGYECQPIFLNVLEAIEPGVVCAGHDNNQPDSFAALLSSLNELGERQLVHVVKWAKALPGFRNLHVDDQMAVIQYSWMGLMVFAMGWRSFTNVNSRMLYFAPDLVFNEYRMHKSRMYSQCVRMRHLSQEFGWLQITPQEFLCMKALLLFSIIPVDGLKNQKFFDELRMNYIKELDRIIACKRKNPTSCSRRFYQLTKLLDSVQPIARELHQFTFDLLIKSHMVSVDFPEMMAEIISVQVPKILSGKVKPIYFHTQ

SEQ ID NO: 3 - DNA, 10063 bp, Mus musculus
cagcgccccctcggagatccctaggagccagcctgctgggagaaccagagggtccggagcaaacctggaggctgagagggcatcagaggggaaaagactgagctagccactccagtgccatacagaagcttaagggacgcaccacgccagccccagcccagcgacagccaacgcctgttgcagagcggcggcttcgaagccgccgcccaggagctgccctttcctcttcggtgaagtttctaaaagctgcgggagactcagaggaagcaaggaaagtgtccggtaggactacggctgcctttgtcctcttcccctctacccttaccccctcctgggtcccctctccaggagctgactaggcaggctttctggccaaccctctcccctacacccccagctctgccagccagtttgcacagaggtaaactccctttggctgagagtaggggagcttgttgcacattgcaaggaaggcttttgggagcccagagactgaggagcaacagcacgcccaggagagtccctggttccaggttctcgcccctgcacctcctcctgcccgcccctcaccctgtgtgtggtgttagaaatgaaaagatgaaaaggcagctagggtttcagtagtcgaaagcaaaacaaaagctaaaagaaaacaaaaagaaaatagcccagttcttatttgcacctgcttcagtggactttgaatttggaaggcagaggatttccccttttccctcccgtcaaggtttgagcatcttttaatctgttcttcaagtatttagagacaaactgtgtaagtagcagggcagatcctgtcttgcgcgtgccttcctttactggagactttgaggttatctgggcactccccccacccaccccccctcctgcaagttttcttccccggagcttcccgcaggtgggcagctagctgcagatactacatcatcagtcaggagaactcttcagagcaagagacgaggaggcaggataagggaattcggtggaagctacagacaagctcaaggatggaggtgcagttagggctgggaagggtctacccacggcccccatccaagacctatcgaggagcgttccagaatctgttccagagcgtgcgcgaagcgatccagaacccgggccccaggcaccctgaggccgctaacatagcacctcccggcgcctgtttacagcagaggcaggagactagcccccggcggcggcggcggcagcagcacactgaggatggttctcctcaagcccacatcagaggccccacaggctacctggccctggaggaggaacagcagccttcacagcagcaggcagcctccgagggccaccctgagagcagctgcctccccgagcctggggcggccaccgctcctggcaaggggctgccgcagcagccaccagctcctccagatcaggatgactcagctgccccatccacgttgtccctgctgggccccactttcccaggcttaagcagctgctccgccgacattaaagacattttgaacgaggccggcaccatgcaacttcttcagcagcagcaacaacagcagcagcaccaacagcagcaccaacagcaccaacagcagcaggaggtaatctccgaaggcagcagcgcaagagccagggaggccacgggggctccctcttcctccaaggatagttacctagggggcaattcaaccatatctgacagtgccaaggagttgtgtaaagcagtgtctgtgtccatgggattgggtgtggaagcattggaacatctgagtccaggggaacagcttcggggagactgcatgtacgcgtcgctcctgggaggtccacccgcggtgcgtcccactccttgtgcgccgctgcccgaatgcaaaggtcttcccctggacgaaggcccaggcaaaagcactgaagagactgctgagtattcctctttcaagggaggttacgccaaaggattggaaggtgagagcttggggtgctctggcagcagtgaagcaggtagctctgggacacttgagatcccgtcctctctgtctctgtataaatctggagcactagacgaggcagcagcataccagaatcgcgactactacaactttccgctggctctgtccgggccgccgcaccccccgccccctacccatccacacgcccgtatcaagctggagaacccattggactacggcagcgcctgggctgcggcggcagcgcaatgccgctatggggacttgggtagtctacatggagggagtgtagccgggcccagcactggatcgcccccagccaccacctcttcttcctggcatactctcttcacagctgaagaaggccaattatatgggccaggaggcgggggcggcagcagcagcccaagcgatgccgggcctgtagccccctatggctacactcggccccctcaggggctgacaagccaggagagtgactactctgcctccgaagtgtggtatcctggtggagttgtgaacagagtaccctatcccagtcccaattgtgtcaaaagtgaaatgggaccttggatggagaactactccggaccttatggggacatgcgtttggacagtaccagggaccatgttttacccatcgactattactttccaccccagaagacctgcctgatctgtggagatgaagcttctggctgtcactacggagctctcacttgtggcagctgcaaggtcttcttcaaaagagccgctgaagggaaacagaagtatctatgtgccagcagaaacgattgtaccattgataaatttcggaggaaaaattgcccatcttgtcgtctccggaaatgttatgaagcagggatgactctgggagctcgtaagctgaagaaacttggaaatctaaaactacaggaggaaggagaaaactccaatgctggcagccccactgaggacccatcccagaagatgactgtatcacacattgaaggctatgaatgtcagcctatctttcttaacgtcctggaagccattgagccaggagtggtgtgtgccggacatgacaacaaccaaccagattcctttgctgccttgttatctagcctcaatgagcttggagagaggcagcttgtgcatgtggtcaagtgggccaaggccttgcctggcttccgcaacttgcatgtggatgaccagatggcggtcattcagtattcctggatgggactgatggtatttgccatgggttggcggtccttcactaatgtcaactccaggatgctctactttgcacctgacttggttttcaatgagtaccgcatgcacaagtctcggatgtacagccagtgtgtgaggatgaggcacctgtctcaagagtttggatggctccaaataaccccccaggaattcctgtgcatgaaagcactgctgctcttcagcattattccagtggatgggctgaaaaatcaaaaattctttgatgaacttcgaatgaactacatcaaggaactcgatcgcatcattgcatgcaaaagaaagaatcccacatcctgctcaaggcgcttctaccagctcaccaagctcctggattctgtgcagcctattgcaagagagctgcatcagttcacttttgacctgctaatcaagtcccatatggtgagcgtggactttcctgaaatgatggcagagatcatctctgtgcaagtgcccaagatcctttctgggaaagtcaagcccatctatttccacacacagtgaagatttggaaaccctaatacccaaaacccaccttgttccctttccagatgtcttctgcctgttatataactctgcactacttctctgcagtgccttgggggaaattcctctactgatgtacagtctgtcgtgaacaggttcctcagttctatttcctgggcttctccttctttttttttcttcttccctccctctttcaccctcccatggcacattttgaatctgctgcgtattgtggctcctgcctttgttttgatttctgttgtatttctttgaatctgtgatgatcctcttgtggcccagtgtcaattgtgcttgtttatagcactgtgctgtgtgccaaccaagcaaatgtttactcaccttatgccatggcaaatttagagagctataagtatctggagaagaaacaaacagagagaataaaaagcaaaaacaaaaccaaaaaataaaaaaaacacaaacaaaaaacaaaaccaacaaacaaaacatgctaggtttgtttcttcgtggtatacaaataaacacataggattcccaaagaagccgacagtgactagaagaaagtaaaaaattacaaatccacgaggagtcactgtttttgttcatcctgtttctctgtgggaaacttcagttgttgttaatggctattgccattaaagagcaggttgaccccaaagctttactgatagggtagagagaaaagaggacaaggagggcagatggataaccattacctccccacagcctttgtccctgagtcctagagtgctcagttgcagtgtagttccttgtactgaaatgtgcttcttgtttgaaaacttgtctgcatgtgaatgcctcttccttccaatccttttctctcttaacctctgcttccaccctcaattgactttcaatagcttttctcagagctttgtactatatgctctctttagccaaaacttggccactttcactgaagttatgtcagtgagaagaaagtggaaaggtctgactctttggaaggctctattcagatttatgttcatatttccatgtgtgagccatagcggagctttgtgactggagtcagaggaaaaggaagtgatggcttagccattctcccattagagatagtgaatgatgatgccatagtgcaatcatcctttcctctgcttttaaaggacctagagaccccatgcagccacattctccctgcacaagtcttcagtgttcagtggccctgaacttcaccaaaatgcatttaagccaaggtggtaaagcttgtacacttctttggacgtgtttgtagacactgctaagatctccctctcaccaccaccacaaaggctagcaggccagcagccacagcatctatgtttagatgttaatagcataaaagacatctcactcaatgtctttcatcaacagtaaatttctggagcccttagaaaaattggaaagaaagcatcaaagggaccagacaaaatgggcatcttgcccttgtcctccagagacaatatattcctcccaagtggagaaatgtcaatttcctcctcagaacaattaaaggggctacccagaccatggtggaagagaaaactaagtaacccagctgagaaaaatgaagacactagaaccagaaagcacaggactttttcctttccatccagcatacccattggcagaaataatggaaggaaaagagaaggccagaagaaaatacagactgctgaagtcttcagaggcaaagtctaaagccagatgaataccatctggctagatgggcatcagtttgctcatcctcctctattgccattgctgggctgactttggccaaagttacttcgaatctccaccatagttgtcccctctcagtcagagggtgcaggaccactgaaacattctatccaccgtgactctcattggacagatctggccggtgtggctacaaatagactgcacccataaactcagggcaagccctgggtcactggtttcatgtagtctgttgacagccttctttactgtggactctgttcctcaaccttgagtgcaggaggaatgcacatctacttttgcctttgtatcattcctcctcactcagctcttcacctccctgcagaccttaagaaatcaggggccagctgccaagctgactcttttggttggtactatgttaactgaaaaggtgatttccgaaggacaggttttcttccctgatttctttgttgctattaatagcaaaaacaaacttgcaaaacaacttctttaacaaggaagggaggatatatacaatgggtgatatggtaatccaaccctgcttgacaaaaactgaagctgacaggttacatttaaaaacaaaacaaaacaaaacgggacagtttctgatttgctttgtgacaacaccatctggcttatgtacaggagctctcttagctgttccttaaacagaaaaaaaatcattactccttttagttaaatttggttacattttaatagtttctttacatctattctgaagcaatttttgtcttctgtggtacatggattttattataacattctaatatttgtctttgtaaatactagagactctttgatccatttctctaggaagtttttcatcttatggagttctgaatcatgacttttatctttatgaatgtatatgctttttacttgcaaaagccaaaaagagtgaaacagcagtgcaattaaagcaacaccaactaaactccaaatttccaagtgacaatattagagaaaaacagcatacacatggctttatgcctactgcttctgcggtggggtttgggtgcgcaatggaaactgtagcttggctgtgttctcccacacaagtgaagaagagattggtttttgcttttttggattttgtgtttcttttctgttttgttttgttttgttttgttttgctttgctttctttggccatcaatgttccaactaatatgattggcggagcacgtgctctgctcagtagagtgaatgttgctggtgcactatgctcacctgtgaacggctggccatttctccattcatatggttaagatggaagatgaggatcacttaccagagaagtcaaggtgatcatctccaaagaggtttacagtgcttggtaggaatggaaaatgaggacaagaaaaagaggagaaccatggagaaggcccaactgggcaggacagcagccagctgccaaagtcacgaactctgggattcaagaagagtcgtgtagtgctttcaactctcatccgcaggcagctcactgtgtgtggactctgagctgacacgggagttggcttctttgttccatagattttctatgccacaggcaatattattgttcttggaaagttcattatttttttaaattaccttactctcagaaagggatttttttgaaggattctgtcatatatctttggaaaacagaaaatcagtaatatgtatatttttatgtatgttcactggcactaaaaaaaaaaaaaaaaagaaaagaaaaaaaagagaaaaaaaaaagcttcactctgtcctttgggtagttgctgaggttaattgtccaggttgagaaatgtgcttctgctaacatccttctctgtccacactctatttctaagtacatataggcatatataggaagatatattcaacacactttaagaaaaaagtatgtccaccatccacatgataaccacaatgatactccacaaattacatgactttaagcttcaagcaacttctaactgattcattcatttatagccttgccctcttctttcccttaaatttggcccagcacaaagacccaagccacccttatacctccctaagacttaagccagcaccagacttcagaaggttttctgaagacaactgacttgctatccctgcatgaccctagcatggtcctgcaaacacaagagactaattataattctcctccactaattgcctgggtcacaggtcattgggccaaggccatgattcttatgcttacgaaccactaatgctaacctactagattaaatcctgaactgaaagttaaaagaagccatttagcatgtgaaacttcttggagtaagaagtttctgtcccggctgcctttgcaaacaggtttgctttcaccacttatctccttgaaaatctttgaaggccttttttttttaagtagaaaaggagatgaaagcattatattatgtaaccaaagattatattgtatctaagataccaaattttttaagggcagggaaggagcaagcattagtgcctctttggtaaattatccaaagacagactgaaggacttttctgatgattgacttagaagactttgtggggaggggttgtctcacaatatacatatttagaagtgttgagaataatttggggggaaatgggattatagtgtccttcactaactgattttataagcagaactagctttccttttttttttttttaaagtagttacaaagcaaattcttaaagctccatctttgcatggttagaaatggagctggtcttggccactgtgtttactagtgcccatgttagcttatttgaagatgtgaagcccttgataagaaggggtacatttaaaggattagatttttgcactagaaggagggcaggcagaaaccctcatttctgcccagtttggacagcacaaaaagttctctgcagtttaaggcagaaagttgaaatatattgtaaatgagtatttgtatccatgtttcaaaactgaattctatatatagatgtaatgtgttctgatagctttacctttctctgcacctttatatttggttccaggtcatatctgatgccatgtacttgtaagagaggttgcagttacatttttggatgctctctcagaatggataagacacctggattgatcagataactgagatctcttcccttcttgggcctggtgttgaggccttgcaaaggggtggaagaggaaagggtagggtacatgatgtattgcactttactagcttaagacggatgaatgtggaaagggtggtgaaatttcattgaaaatgcctaggaattgcaatagggagaaatccagatgtggggccaggtgcccacccaaaggactggccagcagcctcttcatgggatctgaggcattgggaaaaggaaggctatttccttggttttcaccatccttgttagagaagggcagttgcctggtcttgggaacctggagcaaacgctccttctgtcacatcaattctttcccctgcaattgaggtgctcttgctactgggtgtccgtgtgctctaattctggttctggatatgttctgtaaagattttgataattgctaatgtatttttctctgttaaaaatttgttagtgtgttagaagtcatatctctgtaggtacagatcctttgctacccatgagtagagggattttttttcttcaattaagagtttgaccctggggtctgttgcccagagcccatccagaaaaaaaaatccacatttgtcacaatttttctgaaatttcagtcaaggtaacagatcgctgggagttctctttacccccccaaaaaagcagataattgaatttagcaggtggtgttttagagcaaaaaacaaaacagcctttgacccagctttaatatgacccaatttaatctggccaggaagcaggtaatgtgtattaattggcttccaatcctggttgagtgtagcaaggttctactttgtttcctagttccttttgttacatggcctttcacagaaaggattgactgggtttgcagtatatcttatggccttagcacctattgctaactgtcctgaagggaattgcctatggggttgtcctataagccacttctatcattaaaagcagccaccaatggaatctcccaggtttgaaaaaaaaaaaaaaaaacagatggtcctttaccattcattgacacacatccctgctttcctgtagacagattgactggacattgattagggaatacatggcaaatgacatgcttacactaccctggagattaatttggcagtaggagggaatagacaatgtaaccaagaatgtaatgtaattcttatagagataagaattaaatctggatgtggagagagcaaagagagaaagcattcaatttttttttcaaaagaaaccaatttattttgcttgaaacttctttcgctggggcttcagttctcacagcggctcttggtctccactgggcagcaggaccagccccaagcgctagtgttctgttctctttttgtaatcttggaatcttttgttgctctaaatacaattaaaaatggcagaaacttgtttgttggaatac

SEQ ID NO: 4 - protein, 899 aa, Mus musculus
MEVQLGLGRVYPRPPSKTYRGAFQNLFQSVREAIQNPGPRHPEAANIAPPGACLQQRQETSPRRRRRQQHTEDGSPQAHIRGPTGYLALEEEQQPSQQQAASEGHPESSCLPEPGAATAPGKGLPQQPPAPPDQDDSAAPSTLSLLGPTFPGLSSCSADIKDILNEAGTMQLLQQQQQQQQHQQQHQQHQQQQEVISEGSSARAREATGAPSSSKDSYLGGNSTISDSAKELCKAVSVSMGLGVEALEHLSPGEQLRGDCMYASLLGGPPAVRPTPCAPLPECKGLPLDEGPGKSTEETAEYSSFKGGYAKGLEGESLGCSGSSEAGSSGTLEIPSSLSLYKSGALDEAAAYQNRDYYNFPLALSGPPHPPPPTHPHARIKLENPLDYGSAWAAAAAQCRYGDLGSLHGGSVAGPSTGSPPATTSSSWHTLFTAEEGQLYGPGGGGGSSSPSDAGPVAPYGYTRPPQGLTSQESDYSASEVWYPGGVVNRVPYPSPNCVKSEMGPWMENYSGPYGDMRLDSTRDHVLPIDYYFPPQKTCLICGDEASGCHYGALTCGSCKVFFKRAAEGKQKYLCASRNDCTIDKFRRKNCPSCRLRKCYEAGMTLGARKLKKLGNLKLQEEGENSNAGSPTEDPSQKMTVSHIEGYECQPIFLNVLEAIEPGVVCAGHDNNQPDSFAALLSSLNELGERQLVHVVKWAKALPGFRNLHVDDQMAVIQYSWMGLMVFAMGWRSFTNVNSRMLYFAPDLVFNEYRMHKSRMYSQCVRMRHLSQEFGWLQITPQEFLCMKALLLFSIIPVDGLKNQKFFDELRMNYIKELDRIIACKRKNPTSCSRRFYQLTKLLDSVQPIARELHQFTFDLLIKSHMVSVDFPEMMAEIISVQVPKILSGKVKPIYFHTQ

SEQ ID NO: 5 - DNA, 4137 bp, Rattus norvegicus
atccctaggagccagcctgctgggagaaccagagggtccggagcaaacctggaggctgagagggcatcagaggggaaaagactgagttagccactccagtgccatacagaagcttaagggacataccacgccagccccagcccagcgacagccaacgcctgttgcagagcggcggcttcgaagccgccgcccagaagctgccctttcctcttcggtgaagtttctaaaagctgcgggagactcggaggaagcgaagaaagtgtccggtaggactacgactgcctttgtcctcctccctcctacccctacccctcctgggtcccctctccctgagcggactaggcaggcttcctggccagccctctcccctacaccaccagctctgccagccagtttgcacagaggtaactccctttggctgaaagcagacgagcttgttgcccattggaagggaggcttttgggagcccagagactgaggagcaacagcacgctggagagtccctgattccaggttctcccccctgcacctcctactgcccgcccctcaccctgtgtgtgcagctagaattgaaaagatgaaaagacagttggggcttcagtagtcgaaagcaaaacaaaagcaaaaagaaaacaaaaagaaaatagcccagttcttatttgcacctgcttcagtggacattgactttggaaggcagagaattttccttccccccagtcaagctttgagcatcttttaatctgttcttcaagtatttagggacaaactgtgaaactagcagggcagatcctgtctagcgcgtgccttcctttacaggagactttgaggctatctgggcgctcccccccctccctgcaagttttcttccctggagcttcccgcaggtgggcagctagctgcagatactacatcatcagtcagtagaactcttcagagcaagagacgaggaggcaggataagggaattcggtggaagctagagacaagctaaaggatggaggtgcagttagggctgggaagggtctacccacggcccccgtccaagacctatcgaggagcgttccagaatctgttccagagcgtgcgcgaagcgatccagaacccgggccccaggcaccctgaggccgctagcatagcacctcccggtgcctgtttacagcagcggcaggagactagcccccggcggcggcggcggcagcagcaccctgaggatggctctcctcaagcccacatcagaggcaccacaggctacctggccctggaggaggaacagcagccttcacagcagcagtcagcctccgagggccaccctgagagcggctgcctcccggagcctggagctgccacggctcctggcaaggggctgccgcagcagccaccagctcctccagatcaggatgactcagctgccccatccacgttgtccctactgggccccactttcccaggcttaagcagctgctccgcagacattaaagacatcctgagcgaggccggcaccatgcaacttcttcagcagcagcagcaacagcaacagcagcagcagcagcagcagcagcagcagcagcaacagcagcaggaggtaatatccgaaggcagcagcagcgtgagagcaagggaggccactggggctccctcttcctccaaggatagttacctagggggcaattcgaccatatctgacagtgccaaggagttgtgtaaagcagtgtctgtgtccatggggttgggtgtggaagcactggaacatctgagtccaggggagcagcttcggggcgactgcatgtacgcgtcgctcctgggaggtccacccgccgtgcgtcccactccttgtgcgcctctggccgaatgcaaaggtctttccctggacgaaggcccgggcaaaggcactgaagagactgctgagtattcctctttcaagggaggttacgccaaagggttggaaggtgagagtctgggctgctctggcagcagtgaagcaggtagctctgggacacttgagatcccgtcctcactgtctctgtataagtctggagcagtagacgaggcagcagcataccagaatcgcgactactacaactttccgctcgctctgtccgggccgccgcaccccccgccccctacccatccacacgcccgcatcaagctggagaacccgtcggactacggcagcgcctgggctgcggcggcagcgcaatgccgctatggggacttggctagcctacatggagggagtgtagccggacccagcactggatcgcccccagccaccgcctcttcttcctggcatactctcttcacagctgaagaaggccaattatatgggccaggaggcgggggcggcagcagtagcccaagcgatgctgggcctgtagccccctatggctacactcggccccctcaggggctggcaagccaggagggtgacttctctgcctctgaagtgtggtatcctggtggagttgtgaacagagtcccctatcccagtcccagttgtgttaaaagtgaaatgggaccttggatggagaactactccggaccttatggggacatgcgtttggacagtaccagggaccacgttttacccatcgactattacttcccaccccagaagacctgcctgatctgtggagatgaagcttctggttgtcactacggagctctcacttgtggcagctgcaaggtcttcttcaaaagagctgcggaagggaaacagaagtatctatgtgccagcagaaatgattgcaccattgataaatttcggaggaaaaattgtccatcgtgtcgtctccggaaatgttatgaagcagggatgactctgggagctcgtaagctgaagaaacttggaaatctcaaactacaggaagaaggagaaaactccagtgctggtagccccactgaggacccatcccagaagatgactgtatcacacattgaaggctatgaatgtcaacctatctttcttaatgtcctggaagccattgagccaggagtggtgtgtgccggacatgacaacaaccagcctgattcctttgctgccttgttatctagtctcaacgagcttggcgagagacagcttgtacatgtggtcaagtgggccaaggccttgcctggcttccgcaacttgcatgtggatgaccagatggcagtcattcagtattcctggatgggactgatggtatttgccatgggttggcggtccttcactaatgtcaactctaggatgctctactttgcacctgacctggttttcaatgagtatcgcatgcacaagtctcgaatgtacagccagtgcgtgaggatgaggcacctttctcaagagtttggatggctccagataaccccccaggaattcctgtgcatgaaagcactgctactcttcagcattattccagtggatgggctgaaaaatcaaaaattctttgatgaacttcgaatgaactacatcaaggaacttgatcgcatcattgcatgcaaaagaaaaaatcccacatcctgctcaaggcgcttctaccagctcaccaagctcctggattctgtgcagcctattgcaagagagctgcatcaattcacttttgacctgctaatcaagtcccatatggtgagcgtggactttcctgaaatgatggcagagatcatctctgtgcaagtgcccaagatcctttctgggaaagtcaagcccatctatttccacacacagtgaagatttggaaaccctaatacccaaacccaccttgttcccttttcagatgtcttctgcctgttatataactctgcactacttctctggcatgggccttgggggaaattcctctactgatgtacagtctgtcatgaacatgttccccaagttctatttcctgggcttttccttctttctttttcttcttctctgcctcttttaccctcccatggcacattttgaatccgctgcgtgttgtggctcctgcctgtgttttgagttttgttgtatttcttcaagtctgtgatgatcttcttgtggcccagtgtcaactgtgcttgtttatagcactgtgctgtgtgccaaccaagcaaatgtttactcaccttatgccatggcaagtttagagagctataagtatcttgggaagaaacaaacagagagagtaaaaaaacc

SEQ ID NO: 6 - protein, 902 aa, Rattus norvegicus [sequence omitted]

SEQ ID NO: 7 - DNA, 28 bp, Artificial Sequence
  synthetic
acatcaaggaactcgatcgtatcattgc

SEQ ID NO: 8 - DNA, 20 bp, Artificial Sequence
  synthetic
ttgggcacttgcacagagat

SEQ ID NO: 9 - protein, 9 aa, Homo sapiens
LLLFSIIPV

SEQ ID NO: 10 - protein, 10 aa, Homo sapiens
RMLYFAPDLV

SEQ ID NO: 11 - protein, 9 aa, Homo sapiens
FLCMKALLL

SEQ ID NO: 12 - protein, 9 aa, Homo sapiens
QLTKLLDSV

SEQ ID NO: 13 - DNA, 32 bp, Artificial Sequence
  synthetic
ccatcttgtcgtcttcggaaatgttatgaagc

SEQ ID NO: 14 - DNA, 26 bp, Artificial Sequence
  synthetic
tttgaatgaggcaagtcagcctttct

SEQ ID NO: 15 - DNA, 26 bp, Artificial Sequence
  synthetic
tcatgaagtgtgacgttgacatccgt

SEQ ID NO: 16 - DNA, 26 bp, Artificial Sequence
  synthetic
cttagaagcatttgcggtgcacgatg

SEQ ID NO: 17 - DNA, 20 bp, Artificial Sequence
  synthetic
ggaccatgttttacccatcg

SEQ ID NO: 18 - DNA, 20 bp, Artificial Sequence
  synthetic
atctggtcatccacatgcaa

SEQ ID NO: 19 - DNA, 20 bp, Artificial Sequence
  synthetic
ttgttgtggcagcagagttc

SEQ ID NO: 20 - DNA, 19 bp, Artificial Sequence
  synthetic
aagtggggaaccacagcat